European Patent Application EP 4 299 588 A2, published January 3, 2024. Title: TREATMENT METHODS FOR EYE DISORDERS. Applicant: University of Pittsburgh - Of the Commonwealth System of Higher Education. The sequence listing filed with the application follows.

SEQUENCE LISTING (19 sequences)

SEQ ID NO: 1 - DNA, 66 bp, synthetic construct
  misc_feature 1..66: note = Synthetic
  source 1..66: mol_type = other DNA
agctgcaccagatggagacccagactgtgcagcgggagctggaaactcttccaaccaccaagatgg

SEQ ID NO: 2 - protein, 19 aa, synthetic construct
  REGION 1..19: note = Synthetic
METQTVQRELETLPTTKMA

SEQ ID NO: 3 - DNA, 70 bp, synthetic construct
  misc_feature 1..70: note = Synthetic
  source 1..70: mol_type = other DNA
agctgcaccagccaccatggagacccagactgtgcagcggagctggaaactcttccaaccaccaagatgg

SEQ ID NO: 4 - protein, 19 aa, synthetic construct
  REGION 1..19: note = Synthetic
METQTVQRELETLPTTKMA

SEQ ID NO: 5 - DNA, 66 bp, synthetic construct
  misc_feature 1..66: note = Synthetic
  source 1..66: mol_type = other DNA
agctgcaccaggtggagacgcagactgtgcagcgggagctggaaactcttccaaccaccaagatgg

SEQ ID NO: 6 - protein, 19 aa, synthetic construct
  REGION 1..19: note = Synthetic
METQTVQRELETLPTTKMA

SEQ ID NO: 7 - protein, 33 aa, synthetic construct
  REGION 1..33: note = Synthetic DARPin consensus sequence
  REGION 2..3: note = MISC_FEATURE - Xaa is any amino acid except Cys, Pro or Gly
  SITE 5: note = MISC_FEATURE - Xaa is any amino acid except Cys, Pro or Gly
  REGION 13..14: note = MISC_FEATURE - Xaa is any amino acid except Cys, Pro or Gly
  SITE 26: note = MISC_FEATURE - Xaa is His, Asp or Tyr
  SITE 33: note = MISC_FEATURE - Xaa is any amino acid except Cys, Pro or Gly
DXXGXTPLHLAAXXGHLEIVEVLLKXGADVNAX

SEQ ID NO: 8 - DNA, 99 bp, synthetic construct
  misc_feature 1..99: note = Synthetic reverse translation of DARPIN consensus sequence to a 99 base sequence of most likely codons
  misc_feature 4..9: note = n is A, T, G or C without yielding Cys, Pro or Gly
  misc_feature 13..15: note = n is A, T, G or C without yielding Cys, Pro or Gly
  misc_feature 37..42: note = n is A, T, G or C without yielding Cys, Pro or Gly
  misc_feature 97..99: note = n is A, T, G or C without yielding Cys, Pro or Gly
  source 1..99: mol_type = other DNA
gatnnnnnnggcnnnaccccgctgcatctggcggcgnnnnnnggccatctggaaattgtggaagtgctgctgaaataaggcgcggatgtgaacgcgnnn

SEQ ID NO: 9 - DNA, 603 bp, synthetic construct
  misc_feature 1..603: note = Synthetic IFNL1 interferon lambda 1
  source 1..603: mol_type = other DNA
atggctgcagcttggaccgtggtgctggtgactttggtgctaggcttggccgtggcaggccctgtccccacttccaagcccaccacaactgggaagggctgccacattggcaggttcaaatctctgtcaccacaggagctagcgagcttcaagaaggccagggacgccttggaagagtcactcaagctgaaaaactggagttgcagctctcctgtcttccccgggaattgggacctgaggcttctccaggtgagggagcgccctgtggccttggaggctgagctggccctgacgctgaaggtcctggaggccgctgctggcccagccctggaggacgtcctagaccagccccttcacaccctgcaccacatcctctcccagctccaggcctgtatccagcctcagcccacagcagggcccaggccccggggccgcctccaccactggctgcaccggctccaggaggcccccaaaaaggagtccgctggctgcctggaggcatctgtcaccttcaacctcttccgcctcctcacgcgagacctcaaatatgtggccgatgggaacctgtgtctgagaacgtcaacccaccctgagtccacctga

SEQ ID NO: 10 - protein, 200 aa, synthetic construct
  REGION 1..200: note = Synthetic translated amino acid sequence corresponding to SEQ ID NO: 9
MAAAWTVVLVTLVLGLAVAGPVPTSKPTTTGKGCHIGRFKSLSPQELASFKKARDALEESLKLKNWSCSSPVFPGNWDLRLLQVRERPVALEAELALTLKVLEAAAGPALEDVLDQPLHTLHHILSQLQACIQPQPTAGPRPRGRLHHWLHRLQEAPKKESAGCLEASVTFNLFRLLTRDLKYVADGNLCLRTSTHPEST

SEQ ID NO: 11 - DNA, 21 bp, synthetic construct
  misc_feature 1..21: note = Synthetic
  source 1..21: mol_type = other DNA
aggagctagcgagcttcaaga

SEQ ID NO: 12 - DNA, 21 bp, synthetic construct
  misc_feature 1..21: note = Synthetic
  source 1..21: mol_type = other DNA
ggagctagcgagcttcaagaa

SEQ ID NO: 13 - DNA, 21 bp, synthetic construct
  misc_feature 1..21: note = Synthetic
  source 1..21: mol_type = other DNA
gagctagcgagcttcaagaag

SEQ ID NO: 14 - DNA, 21 bp, synthetic construct
  misc_feature 1..21: note = Synthetic
  source 1..21: mol_type = other DNA
agctagcgagcttcaagaagg

SEQ ID NO: 15 - DNA, 21 bp, synthetic construct
  misc_feature 1..21: note = Synthetic
  source 1..21: mol_type = other DNA
gccttggaagagtcactcaag

SEQ ID NO: 16 - DNA, 21 bp, synthetic construct
  misc_feature 1..21: note = Synthetic
  source 1..21: mol_type = other DNA
aggcatctgtcaccttcaacc

SEQ ID NO: 17 - DNA, 21 bp, synthetic construct
  misc_feature 1..21: note = Synthetic
  source 1..21: mol_type = other DNA
ggcatctgtcaccttcaacct

SEQ ID NO: 18 - DNA, 5591 bp, synthetic construct
  misc_feature 1..5591: note = Synthetic scCAG_hCryba1
  misc_feature 3452: note = n is a, c, g, or t
  source 1..5591: mol_type = other DNA
cagcagctgcgcgctcgctcgctcactgaggccgcccgggcaaagcccgggcgtcgggcgacctttggtcgcccggcctcagtgagcgagcgagcgcgcagagagggagtggggttcggtacccgttacataacttacggtaaatggcccgcctggctgaccgcccaacgacccccgcccattgacgtcaataatgacgtatgttcccatagtaacgccaatagggactttccattgacgtcaatgggtggagtatttacggtaaactgcccacttggcagtacatcaagtgtatcatatgccaagtacgccccctattgacgtcaatgacggtaaatggcccgcctggcattatgcccagtacatgaccttatgggactttcctacttggcagtacattactcgaggccacgttctgcttcactctccccatctccccccccctccccacccccaattttgtatttatttattttttaattattttgtgcagcgatgggggcggggggggggggggggcgcgcgccaggcggggcggggcggggcgaggggcggggcggggcgaggcggagaggtgcggcggcagccaatcagagcggcgcgctccgaaagtttccttttatggcgaggcggcggcggcggcggccctataaaaagcgaagcgcgcggcgggcgggagcgggatcagccaccgcggtggcggcctagagtcgacgaggaactgaaaaaccagaaagttaactggtaagtttagtctttttgtcttttatttcaggtcccggatccggtggtggtgcaaatcaaagaactgctcctcagtggatgttgcctttacttctaggcctgtacggaagtgttacttctgctctaaaagctgcggaattgtacccgcggccgatccaccgggccaccatggagacccaggctgagcagcaggagctggaaacccttccaaccaccaagatggctcagaccaaccctacgccggggtccctggggccatggaagataaccatctatgatcaggagaactttcagggcaagaggatggagttcaccagctcctgtccaaatgtctctgagcgcagttttgataatgtccggtccctgaaggtggaaagtggcgcctggattggttatgagcataccagcttctgtgggcaacagtttatcctggagagaggagaataccctcgctgggatgcctggagtgggagtaatgcctaccacattgagcgtctcatgtccttccgccccatctgttcagctaatcataaggagtctaagatgaccatctttgagaaggaaaactttattggacgccagtgggagatctctgacgactacccctccttgcaagccatgggctggttcaacaacgaagtcggctccatgaagatacaaagtggggcctgggtttgctaccaatatcctggatatcgtgggtatcagtatatcttggaatgtgaccatcatggaggagactataaacattggagagagtggggctctcatgcccagacttcgcagatccaatcgattcgccgaatccaacagtagagctcgctgatcagcctcgactgtgccttctagttgccagcatctgttgtttgcccctcccccgtgccttccttgaccctggaaggtgccactcccactgtcctttcctaataaaatgaggaaattgcatcgcattgtctgagtaggtgtcattctattctggggggggggtggggcaggacagcaagggggaggattgggaagacaatagcaggctggggagagatcctagtttccatgctctaggagcatggctacgtagataagtagcatggcgggttaatcattaactacaggaacccctagtgatggagttggccactccctctctgcgcgctcgctcgctcactgaggccgggcgaccaaaggtcgcccgacgcccgggctttgcccgggcggcctcagtgagcgagcgagcgcgcagctggcgtaatagcgaagaggcccgcaccgatcgcccttcccaacagttgcgcagcctgaatggcgaatggaattccagacgattgagcgtcaaaatgtaggtatttccatgagcgtttttcctgtgcaatggctggcggtaatattgttctggatattaccagcaaggccgatagtttgagttcttctactcaggcaagtgatgttattactaatcaaagaagtattgcgacaacggttaatttgcgtgatgacagactcttttactcggtggcctcactgattataaaaacacttctcaggattctggcgtaccgttcctgtctaaaatccctttaatcggcctcctgtttagctcccgctctgattctaacgaggaagcacgttatacgtgctcgtcaaagcaaccatagtacgcgccctgtagcggcgcattaagcgcggcgggtgtggtggttacgcgcagcgtgaccgctacacttgccagcgccctagcgcccgctccttcgctttcttcccttcctttctcgccacgttcgccggctttccccgtcaagctctaaatcgggggctccctttagggttccgatttagtgctttacggcacctcgaccccaaaaaacttgattaggggatggttcacgtagtgggccatcgccctgatagacggtttttcgccctttgacgttggagtccacgttctttaatagtggactcttgttccaaactggaacaacactcaaccctatctcggtctattttttgatttataagggattttgccgatttcggcctattggttaaaaaatgagctgatttaacaaaaatttaacgcgaattttaacaaaatattaacgtttacaatttaaatatttgcttatacaatctcctgtttttggggcttttctgattatcaaccggggtacatatgattgacatgctagttttacgattaccgttcatcgattctcttgtttgctccagactctcaggcaatgacctgatagcctttgtgagacctctcaaaaatagctaccctctccggcatgaatttatcagctagaacggttgaatatcatattgatggtgatttgactgtctccggcctttctcacccgtttgaatctttacctacacattatcaggcattgcatttaaaatatatgagggttctaaaaatttttatccttgcgttgaaataaaggcttctcccgcaaaagtattacagggtcataatgtttttggtacaaccgatttagctttatgcttgaggctttattgcttaattttgctaattctttgccttgcctgtatgatttattggatgttggaattcctgatgcggtattttctccttacgcatctgtgcggtatttcacaccgcatatggtgcacctcagtacaatctgctctgatgccgcatagttaagccagccccgacacccgccaacacccgctgacgcgccctngacgggcttgtctgctcccggcatccgcttacagacaagctgtgaccgtctccgggagctgcatgtgtcagaggttttcaccgtcatcaccgaaacgcgcgagacgaaagggcctcgtgatacgccttttttataggttaatgtcatgataataatggtttcttagacgtcaggtggcacttttcggggaaatgtgcgcggaacccctatttgtttatttttctaaatacattcaaatatgtatccgctcatgaacaataaccctgataaatgcttcaataatattgaaaaaggaagagtatgagtattcaacatttccgtgtcgcccttattcccttttttgcggcattttgccttcctgtttttgctcacccagaaacgtggtgaaagtaaaagatgctgaagatcagttgggtgcacgagtgggttacatcgaactggatctcaacagcggtaagatccttgagagttttcgccccgaagaacgttttccaatgatgagcactttaaagttctgctatgtggcgcggtattatcccgtattgacgccgggcaagagcaactcggtcgccgcatacactattctcagaatgacttggttgagtactcaccagtcacagaaaagcatcttacggtggcatgacagtaagagaattatgcagtgctgccataaccatgagtgataacactgcggccaacttacttctgacaacgatcggaggaccgaaggagctaaccgcttttttgcacaacatgggggatatgtaactcgccttgatcgttgggaaccggagctgaatgaagccataccaaacgacgagcgtgacaccacgatgcctgtagcaatggcaacaacgttgcgcaaactattaactggcgaactacttacctagcttcccggcaacaattaatagactggatggaggcggataaagttgcaggaccacttctgcgctcggcccttccggctggctggtttattgctgataaatctggagccggtgagcgtgggtctccggtatcattgcagcactggggccagatggtaagccctcccgtatcgtagttatctacacgacggggagtcaggcaactatggatgaacgaaatagacagatcgctgagataggtgcctcactgattagcattggtaactgtcagaccaagtttactcatatatactttagattgatttaaaacttcatttttaatttaaaaggatctaggtgaagatcctttttgataatctcatgaccaaaatcccttaacggagttttcgttccactgagcgtcagaccccgtagaaaagatcaaaggatcttcttgagatcctttttttctgcgcgtaatctgctgcttgcaaacaaaaaaaccaccgctaccagcggtggtttgttgccggatcaagagctaccaactctttttccgaaggtaactggcttcagcagagcgcagataccaaatactgtccttctagtgtagccgtagttaggccaccacttcaagaactctgtagcaccgcctcatacctcgctctgctaatcctgttaccagtggctgctgccagtggcgataagtcgtgtcttaccgggttggactcaagacgatagttaccggataaggcgcagcggtcgggctgaacggggggttctgcacacagcccagcttggagcgaacgacctacaccgaactgagatacctacagcgtgagctatgagaaagcgccacgcttcccgaagggagaaaggcggacaggtatccggtaagcggcagggtcgaacaggagagcgcacgagggagcttccagggggaaacgcctggtatctttatagtcctgtcgggtttcgccacctctgacttgagcgtcgatttttgtgatgctcgtcaggggggcggagcctatggaaaacgccagcaacgcggcctttttacggttcctggccttttgctggccttttgctcacatgttctttcctgcgttatcccctgattctgtggataaccgtattaccgcctttgagtgagctgatacgctcgccgcagccgaacgaccgagcgcagcgagtcagtgagcgaggaagcggaagagcgcccaatacgcaaaccgcctctccccgcgcgttggccgattcattaatg

SEQ ID NO: 19 - DNA, 648 bp, synthetic construct
  misc_feature 1..648: note = Synthetic
  source 1..648: mol_type = other DNA
atggagacccagactgtgcagcgggagttggaaactcttccaaccaccaagatggctcagaccaaccctatgccaggatccttggggccatggaagataaccatctacgatcaagagaacttccagggcaagaggatggagttcaccagctcctgcccaaatgtctctgaacgtaattttgataatgtccggtcacttaaggtggagtgtggcgcctggattggttatgaacacaccagcttctgtgggcaacagttcatcctggaaagaggagaataccctcgatgggatgcctggagcgggagcaatgcctatcatattgagcgtctcatgtccttccgacccatctgttccgctaatcataaagagtctaagattaccatcttcgagaaagagaactttattggacgccagtgggaaatctgtgatgactacccttccttgcaagccatgggttggttcaacaatgaagttggttccatgaagatacaatgtggggcctgggtttgctaccagtaccctggatatcgtggttatcagtatatcttggagtgtgaccaccatggaggagactacaagcactggccagagtggggatctcacgcccagacttcccagatccaatcaattcgccgaatacaacaatag